European Patent Specification EP 3 384 075 B1, published September 6, 2023. Title: A METHOD OF RESIDUE PROXIMITY INFORMATION AND PROTEIN MODEL DISCRIMINATION USING SATURATION-SUPPRESSOR MUTAGENESIS. Applicant: INDIAN INSTITUTE OF SCIENCE. The sequence listing filed with the application follows.

SEQUENCE LISTING (2 sequences)

SEQ ID NO: 1 - protein, 101 aa, artificial sequence
  CcdB protein sequence
MQFKVYTYKRESRYRLFVDVQSDIIDTPGRRMVIPLASARLLSDKVSRELYPVVHIGDESWRMMTTDMASVPVSVIGEEVADLSHRENDIKNAINLMFWGI

SEQ ID NO: 2 - protein, 121 aa, artificial sequence
  DgkA protein
ANNTTGFTRIIKAAGYSWKGLRAAWINEAAFRQEGVAVLLAVVIAAWLDVDAITRVLLISSVMLVMIVEILNSAIEAVVDRIGSEYHELSGRAKDMGSAAVLIAIIVAVITWAILLWSHFG